European Patent Application EP 4 368 182 A1, published May 15, 2024. Title: Tau-tubulin kinase (TTBK) inhibitor compounds. Applicant: Consejo Superior de Investigaciones Cientificas (CSIC). The sequence listing filed with the application follows.

SEQUENCE LISTING (1 sequence)

SEQ ID NO: 1 - protein, 18 aa, synthetic construct
  REGION 1..18: note = Peptide used in Example 2; note (original language) = Peptido utilizado en el ejemplo 2
  source 1..18: organism (original language) = Secuencia Artificial
RRKDLHDDEEDEAMSITA